European Patent Application EP 4 438 728 A1, published October 2, 2024. Title: 変異体ライブラリプール作製方法. Applicant: 花王株式会社. The sequence listing filed with the application follows.

SEQUENCE LISTING (14 sequences)

SEQ ID NO: 1 - protein, 286 aa, synthetic construct [sequence omitted]

SEQ ID NO: 2 - DNA, 861 bp, synthetic construct
  source 1..861: mol_type = other DNA; note = beta-lactamase
atgagtattcaacatttccgtgtcgcccttattcccttttttgcggcattttgccttcctgtttttgctcacccagaaacgctggtgaaagtaaaagatgctgaagatcagttgggtgcacgagtgggttacatcgaactggatctcaacagcggtaagatccttgagagttttcgccccgaagaacgttttccaatgatgagcacttttaaagttctgctatgtggcgcggtattatcccgtgttgacgccgggcaagagcaactcggtcgccgcatacactattctcagaatgacttggttgagtactcaccagtcacagaaaagcatcttacggatggcatgacagtaagagaattatgcagtgctgccataaccatgagtgataacactgcggccaacttacttctgacaacgatcggaggaccgaaggagctaaccgcttttttgcacaacatgggggatcatgtaactcgccttgatcgttgggaaccggagctgaatgaagccataccaaacgacgagcgtgacaccacgatgcctgcagcaatggcaacaacgttgcgcaaactattaactggcgaactacttactctagcttcccggcaacaattaatagactggatggaggcggataaagttgcaggaccacttctgcgctcggcccttccggctggctggtttattgctgataaatctggagccggtgagcgtgggtctcgcggtatcattgcagcactggggccagatggtaagccctcccgtatcgtagttatctacacgacggggagtcaggcaactatggatgaacgaaatagacagatcgctgagataggtgcctcactgattaagcattggtaa

SEQ ID NO: 3 - DNA, 35 bp, synthetic construct
  source 1..35: mol_type = other DNA
cttcctgtttttgctnnkccagaaacgctggtgaa

SEQ ID NO: 4 - DNA, 24 bp, synthetic construct
  source 1..24: mol_type = other DNA
agcaaaaacaggaaggcaaaatgc

SEQ ID NO: 5 - protein, 483 aa, synthetic construct
  source 1..483: note = YR288dRT
AAQNGTMMQYFEWYVPNDGQHWNRLRNDAAYLKSIGVSAIWTPPAYKGTSQNDVGYGAYDLYDLGEFNQKGTIRTKYGTKAELKSAVSTLKSNGIQVYGDVVMNHKGGADYTENVTAVEVNPSNRNQETSDEYTIQAWTGFNFPGRGTTHSPFKWQWYHFDGTDWDQSRNASRIFKFGGKAWDWEVSSENGNYDYLMYADLDFDHPDVRNEMKNWGVWYANEVGLDGFRLDAVKHIKHSYLGDWVNHVRTKTGKEMFTVAEYWQNDVNAINNYLAKVNYNHSVFDAPLHYNFHYASQSGGNYDMRNLLNGTVVAAHPTKAVTLVENHDSQPGQSLESVVQPWFKPLAYAFILTRAEGYPSIFYGDMYGTKGNSSYEIPALKTKIEPLLKARKDYAYGTQHNYMDHWDVIGWTREGDSTKEKSGLATLVTDGAGGSKWMYVGKQNAGEVWYDITGNRTDKITINTDGWGNFQVNGGSVSVYVQQ

SEQ ID NO: 6 - DNA, 1449 bp, synthetic construct
  source 1..1449: mol_type = other DNA; note = YR288dRT
gcagctcaaaacggtacgatgatgcagtactttgaatggtatgtaccgaatgatggtcagcattggaatcgtctgcggaacgatgcagcctacttgaaatccatcggtgtgtcagctatctggacacctcctgcttacaaaggcacaagccagaacgatgttggctatggagcatatgacctgtacgatttaggagaattcaaccagaaaggcactattcgcaccaaatatggaacgaaagctgaactgaaaagcgcggtatcgactctcaagtctaatgggattcaagtgtatggagatgtcgtcatgaatcataaaggcggtgccgattacacagagaatgtaacagctgtggaagtcaatccgagcaatcgcaatcaagaaacatccgatgagtatacgatccaagcatggacaggattcaacttccctgggcgaggcacaacccatagtccgtttaagtggcagtggtatcattttgatggaactgactgggatcagtctcggaatgcgagcagaatcttcaaatttgggggaaaagcatgggattgggaagtatcatcggagaatgggaattacgactatcttatgtacgccgatttagactttgatcatcctgatgttagaaatgagatgaagaattggggcgtgtggtacgcgaatgaagttggcttggacggatttaggctggatgcggttaagcacataaagcatagctatctgggcgattgggtgaaccatgtcagaactaagacgggaaaagagatgtttacagttgctgaatattggcaaaacgacgtcaatgccattaataactatttagccaaagtgaactataatcactctgtctttgatgcgcctttgcattacaactttcactatgcaagccagtcaggaggtaactacgacatgcgtaacttattgaacggcacagtcgtggctgctcatccgacaaaagcagttacccttgtcgaaaatcatgacagtcaaccgggacaatctctggagtcagtcgttcaaccgtggtttaagccccttgcctatgcgtttatcctcacacgagcagaaggttatccaagtatcttttatggggatatgtatgggactaagggaaactcatcgtacgaaattccagcactcaaaaccaaaattgaaccgttactgaaagcacgcaaggattatgcctatggtacgcagcacaactatatggaccactgggatgttataggttggaccagagaaggtgactccacgaaagaaaaatctggccttgcgacgcttgtgacagacggggcaggcgggtctaaatggatgtatgtaggcaaacagaatgctggcgaagtttggtatgacatcacaggcaatagaacggataaaatcaccattaatacagatggctggggaaacttccaagtaaacggaggctcagtctccgtgtacgttcaacag

SEQ ID NO: 7 - DNA, 25 bp, synthetic construct
  source 1..25: mol_type = other DNA
tgagatccggctgctaacaaagccc

SEQ ID NO: 8 - DNA, 18 bp, synthetic construct
  source 1..18: mol_type = other DNA
ggccatcgccggctgggc

SEQ ID NO: 9 - DNA, 42 bp, synthetic construct
  source 1..42: mol_type = other DNA
cagccggcgatggccgcagctcaaaacggtacgatgatgcag

SEQ ID NO: 10 - DNA, 41 bp, synthetic construct
  source 1..41: mol_type = other DNA
agcagccggatctcactgttgaacgtacacggagactgagc

SEQ ID NO: 11 - DNA, 35 bp, synthetic construct
  source 1..35: mol_type = other DNA
ggtacgatgatgcagnnktttgaatggtatgtacc

SEQ ID NO: 12 - DNA, 24 bp, synthetic construct
  source 1..24: mol_type = other DNA
ctgcatcatcgtaccgttttgagc

SEQ ID NO: 13 - DNA, 25 bp, synthetic construct
  source 1..25: mol_type = other DNA
gcgaaattaatacgactcactatag

SEQ ID NO: 14 - DNA, 20 bp, synthetic construct
  source 1..20: mol_type = other DNA
gccaatccggatatagttcc